European Patent Application EP 4 763 221 A1, published June 24, 2026. Title: 化合物以及含有该化合物的抗体偶联药物. Applicant: 中山康方生物医药有限公司. The sequence listing filed with the application follows.

SEQUENCE LISTING (16 sequences)

SEQ ID NO: 1 - protein, 8 aa, synthetic construct
  source 1..8: note = HCDR1
GGSFSGYY

SEQ ID NO: 2 - protein, 7 aa, synthetic construct
  source 1..7: note = HCDR2
INHSGST

SEQ ID NO: 3 - protein, 11 aa, synthetic construct
  source 1..11: note = HCDR3
ARDKWTWYFDL

SEQ ID NO: 4 - protein, 12 aa, synthetic construct
  source 1..12: note = LCDR1
QSVLYSSSNRNY

SEQ ID NO: 5 - skipped

SEQ ID NO: 6 - protein, 9 aa, synthetic construct
  source 1..9: note = LCDR3
QQYYSTPRT

SEQ ID NO: 7 - protein, 117 aa, synthetic construct [sequence omitted]

SEQ ID NO: 8 - DNA, 351 bp, synthetic construct
  source 1..351: mol_type = other DNA; note = nucleic acid encoding Patritumab VH
caggtgcagctgcagcagtggggcgccggactgctgaagccatccgagaccctgtctctgacatgtgccgtgtacggcggctccttttctggctactattggagctggatcaggcagccccctggcaagggactggagtggatcggcgagatcaaccacagcggctccaccaactataatccctctctgaagagccgggtgaccatcagcgtggagacatccaagaatcagttctccctgaagctgagctccgtgaccgcagcagacacagccgtgtactattgcgcccgggacaagtggacctggtactttgatctgtggggcagaggcaccctggtgacagtgtctagc

SEQ ID NO: 9 - protein, 113 aa, synthetic construct [sequence omitted]

SEQ ID NO: 10 - DNA, 339 bp, synthetic construct
  source 1..339: mol_type = other DNA; note = nucleic acid encoding Patritumab VL
gacatcgagatgacccagtcccctgattctctggccgtgagcctgggagagagggcaacaatcaactgtagaagctcccagtccgtgctgtactctagctccaaccggaattacctggcctggtatcagcagaatccaggccagccccctaagctgctgatctattgggccagcaccagggagtccggagtgccagaccgcttctccggctctggcagcggcacagacttcaccctgacaatctctagcctgcaggccgaggacgtggccgtgtactattgccagcagtactatagcacccccaggacatttggccagggcaccaaggtggagatcaag

SEQ ID NO: 11 - protein, 330 aa, synthetic construct
  source 1..330: note = Patritumab CH
ASTKGPSVFPLAPSSKSTSGGTAALGCLVKDYFPEPVTVSWNSGALTSGVHTFPAVLQSSGLYSLSSVVTVPSSSLGTQTYICNVNHKPSNTKVDKRVEPKSCDKTHTCPPCPAPELLGGPSVFLFPPKPKDTLMISRTPEVTCVVVDVSHEDPEVKFNWYVDGVEVHNAKTKPREEQYNSTYRVVSVLTVLHQDWLNGKEYKCKVSNKALPAPIEKTISKAKGQPREPQVYTLPPSREEMTKNQVSLTCLVKGFYPSDIAVEWESNGQPENNYKTTPPVLDSDGSFFLYSKLTVDKSRWQQGNVFSCSVMHEALHNHYTQKSLSLSPGK

SEQ ID NO: 12 - DNA, 990 bp, synthetic construct
  source 1..990: mol_type = other DNA; note = nucleic acid encoding Patritumab CH
gcctctacaaaggggcccagcgtgtttcctctggcccctagcagcaagtctacaagcggaggaacagcagctctgggctgcctggtgaaggactacttcccagagcccgtgaccgtgtcttggaactcaggagccctgaccagcggagtgcacacatttccagccgtgctgcagagcagcggactgtatagcctgagcagcgtggtgaccgtgccttcttctagcctgggcacccagacctacatctgcaacgtgaaccacaagcccagcaacaccaaggtggacaagagggtggagcccaagtcttgcgacaagacccacacttgtcctccttgtccagccccagagctgctgggaggaccaagcgtgttcctgttccctcccaagcccaaggacaccctgatgatcagcaggaccccagaagtgacttgcgtggtggtggacgtgtctcacgaggaccccgaagtgaagttcaattggtacgtggacggcgtggaggtgcacaacgctaagaccaagcccagggaggagcagtacaacagcacctaccgggtggtgtccgtgctgacagtgctgcaccaggattggctgaacggcaaggagtacaagtgcaaggtgtccaataaggccctgccagcccctatcgagaagaccatcagcaaggccaagggccagcctagagagcctcaggtgtacaccctgcctccttctcgggaggagatgaccaagaaccaggtgtccctgacttgcctcgtgaagggcttctaccccagcgatattgccgtcgagtgggagtctaacggccagcccgagaacaactacaagaccacacctccagtgctggatagcgacggcagcttcttcctgtacagcaagctgaccgtggacaaaagccgctggcagcagggcaacgtgttttcttgcagcgtgatgcacgaagccctgcacaaccactacacccagaagagcctgagcctgtctccaggcaag

SEQ ID NO: 13 - protein, 107 aa, synthetic construct [sequence omitted]

SEQ ID NO: 14 - DNA, 321 bp, synthetic construct
  source 1..321: mol_type = other DNA; note = nucleic acid encoding Patritumab CL
cgtacggtggcagccccatctgtcttcatttttccccctagtgacgagcagctgaaatccggaacagcctctgtggtctgtctgctgaacaatttctaccctcgcgaagccaaggtgcagtggaaagtcgataacgctctgcagagtggcaattcacaggagagcgtgactgaacaggactccaaggattctacctatagtctgagctccactctgaccctgtccaaagcagattacgaaaagcacaaagtgtatgcctgtgaggtcacccaccaggggctgagttctccagtcaccaaatccttcaacagaggcgaatgt

SEQ ID NO: 15 - protein, 5 aa, synthetic construct
  source 1..5: note = repeat unit of a linker
GGGGS

SEQ ID NO: 16 - protein, 20 aa, synthetic construct
  source 1..20: note = a linker
GGGGSGGGGSGGGGSGGGGS